European Patent Application EP 4 600 343 A1, published August 13, 2025. Title: 超高分子ガンマ－ポリグルタミン酸、該ポリグルタミン酸を産生するバチルス属細菌変異株及び該バチルス属細菌変異株のスクリーニング方法. Applicant: 国立大学法人神戸大学. The sequence listing filed with the application follows.

SEQUENCE LISTING (45 sequences)

SEQ ID NO: 1 - protein, 380 aa, Bacillus subtilis
MKKELSFHEKLLKLTKQQKKKTNKHVFIAIPIVFVLMFAFMWAGKAETPKVKTYSDDVLSASFVGDIMMGRYVEKVTEQKGADSIFQYVEPIFRASDYVAGNFENPVTYQKNYKQADKEIHLQTNKESVKVLKDMNFTVLNSANNHAMDYGVQGMKDTLGEFAKQNLDIVGAGYSLSDAKKKISYQKVNGVTIATLGFTDVSGKGFAAKKNTPGVLPADPEIFIPMISEAKKHADIVVVQSHWGQEYDNDPNDRQRQLARAMSDAGADIIVGHHPHVLEPIEVYNGTVIFYSLGNFVFDQGWTRTRDSALVQYHLKKNGTGRFEVTPIDIHEATPAPVKKDSLKQKTIIRELTKDSNFAWKVEDGKLTFDIDHSDKLKSK

SEQ ID NO: 2 - DNA, 1143 bp, Bacillus subtilis
  source 1..1143: mol_type = other DNA
atgaaaaaagaactgagctttcatgaaaagctgctaaagctgacaaaacagcaaaaaaagaaaaccaataagcacgtatttattgccattccgatcgtttttgtccttatgttcgctttcatgtgggcgggaaaagcggaaacgccgaaggtcaaaacgtattctgacgacgtactctcagcctcatttgtaggcgatattatgatgggacgctatgttgaaaaagtaacggagcaaaaaggggcagacagtatttttcaatatgttgaaccgatctttagagcctcggattatgtagcaggaaactttgaaaacccggtaacctatcaaaagaattataaacaagcagataaagagattcatctgcagacgaataaggaatcagtgaaagtcttgaaggatatgaatttcacggttctcaacagcgccaacaaccacgcaatggattacggcgttcagggcatgaaagatacgcttggagaatttgcgaagcaaaatcttgatatcgttggagcgggatacagcttaagtgatgcgaaaaagaaaatttcgtaccagaaagtcaacggggtaacgattgcgacgcttggctttaccgatgtgtccgggaaaggtttcgcggctaaaaagaatacgccgggcgtgctgcccgcagatcctgaaatcttcatccctatgatttcagaagcgaaaaaacatgcggacattgttgttgtgcagtcacactggggacaagagtatgacaatgatccaaatgaccgccagcgccagcttgcaagagccatgtctgatgcgggagctgacatcatcgtcggccatcacccgcacgtcttagaaccgattgaagtatataacggaaccgtcattttctacagcctcggcaactttgtctttgaccaaggctggacgagaacaagagacagtgcactggttcagtatcacctgaagaaaaatggaacaggacgctttgaagtgacaccgatcgatatccatgaagcgacacctgcgcctgtgaaaaaagacagccttaaacagaaaaccattattcgcgaactgacgaaagactctaatttcgcttggaaagtagaagacggaaaactgacgtttgatattgatcatagtgacaaactaaaatctaaataa

SEQ ID NO: 3 - protein, 393 aa, Bacillus subtilis
MWLLIIACAVILVIGILEKRRHQKNIDALPVRVNINGIRGKSTVTRLTTGILIEAGYKTVGKTTGTDARMIYWDTPEEKPIKRKPQGPNIGEQKEVMRETVERGANAIVSECMAVNPDYQIIFQEELLQANIGVIVNVLEDHMDVMGPTLDEIAEAFTATIPYNGHLVITDSEYTEFFKQKAKERNTKVIIADNSKITDEYLRKFEYMVFPDNASLALGVAQALGIDEETAFKGMLNAPPDPGAMRILPLISPSEPGHFVNGFAANDASSTLNIWKRVKEIGYPTDDPIIIMNCRADRVDRTQQFANDVLPYIEASELILIGETTEPIVKAYEEGKIPADKLHDLEYKSTDEIMELLKKRMHNRVIYGVGNIHGAAEPLIEKIHEYKVKQLVS

SEQ ID NO: 4 - DNA, 1182 bp, Bacillus subtilis
  source 1..1182: mol_type = other DNA
atgtggttactcattatagcctgtgctgtcatactggtcatcggaatattagaaaaacgacgacatcagaaaaacattgatgccctccctgttcgggtgaatattaacggcatccgcggaaaatcgactgtgacaaggctgacaaccggaatattaatagaagccggttacaagactgttggaaaaacaacaggaacagatgcaagaatgatttactgggacacaccggaggaaaagccgattaaacggaaacctcaggggccgaatatcggagagcaaaaagaagtcatgagagaaacagtagaaagaggggctaacgcgattgtcagtgaatgcatggctgttaacccagattatcaaatcatctttcaggaagaacttctgcaggccaatatcggcgtcattgtgaatgttttggaagaccatatggatgtcatggggccgacgcttgatgaaattgcagaagcgtttactgctacaattccttataatggccatcttgtcattacagatagtgaatataccgagttctttaaacaaaaagcaaaagaacgaaacacaaaagtcatcattgctgataactcaaaaattacagatgagtatttacgtaaatttgaatacatggtattccctgataacgcttctctggcgctgggtgtggctcaagcactcggcattgacgaagaaacagcatttaagggaatgctgaatgcgccgccagatccgggagcaatgagaattcttccgctgatcagtccgagcgagcctgggcactttgttaatgggtttgccgcaaacgacgcttcttctactttgaatatatggaaacgtgtaaaagaaatcggttacccgaccgatgatccgatcatcatcatgaactgccgcgcagaccgtgtcgatcggacacagcaattcgcaaatgacgtattgccttatattgaagcaagtgaactgatcttaatcggtgaaacaacagaaccgatcgtaaaagcctacgaagaaggcaaaattcctgcagacaaactgcatgatctagagtataagtcaacagatgaaattatggaattgttaaagaaaagaatgcacaaccgtgtcatatatggcgtcggcaatattcatggtgccgcagagcctttaattgaaaaaatccacgaatacaaggtaaagcagctcgtaagctag

SEQ ID NO: 5 - protein, 149 aa, Bacillus subtilis
MFGSDLYIALILGVLLSLIFAEKTGIVPAGLVVPGYLGLVFNQPVFILLVLLVSLLTYVIVKYGLSKFMILYGRRKFAAMLITGIVLKIAFDFLYPIVPFEIAEFRGIGIIVPGLIANTIQKQGLTITFGSTLLLSGATFAIMFVYYLI

SEQ ID NO: 6 - DNA, 449 bp, Bacillus subtilis
  source 1..449: mol_type = other DNA
tgttcggatcagatttatacatcgcactaattttaggtgtactactcagtttaatttttgcggaaaaaacagggatcgtgccggcaggacttgttgtaccgggatatttaggacttgtgtttaatcagccggtctttattttacttgttttgctagtgagcttgctcacgtatgtcattgtgaaatacggtttatccaaatttatgattttgtacggacgcagaaaattcgctgccatgctgataacagggatcgtcctaaaaatcgcgtttgattttctatacccgattgtaccatttgaaatcgcagaatttcgaggaatcggcatcatcgtgccaggtttaattgccaataccattcagaaacaaggtttaaccattacgttcggaagcacgctgctattgagcggagcgacctttgctatcatgtttgtttactacttaatttaa

SEQ ID NO: 7 - protein, 413 aa, Bacillus subtilis
MNTLANWKKFLLVAVIICFLVPIMTKAEIAEADTSSELIVSEAKNLLGYQYKYGGETPKEGFDPSGLIQYVFSKADIHLPRSVNDQYKIGTAVKPENLKPGDILFFKKEGSTGTVPTHDALYIGDGQMVHSTQSKGVIITNYKKSSYWSGTYIGARRIAADPATADVPVVQEAEKYIGVPYVFGGSTPSEGFDCSGLVQYVFQQALGIYLPRSAEQQWAVGEKVAPQNIKPGDVVYFSNTYKTGISHAGIYAGAGRFIQASRSEKVTISYLSEDYWKSKMTGIRRFDNLTIPKENPIVSEATLYVGEVPYKQGGVTPETGFDTAGFVQYVYQKAAGISLPRYATSQYNAGTKIEKADLKPGDIVFFQSTSLNPSIYIGNGQVVHVTLSNGVTITNMNTSTYWKDKYAGSIRVQ

SEQ ID NO: 8 - DNA, 1242 bp, Bacillus subtilis
  source 1..1242: mol_type = other DNA
gtgaacacactggcaaactggaagaagtttttgcttgtggcggttatcatttgttttttggttccaattatgacaaaagcggagattgcggaagctgatacatcatcagaattgattgtcagcgaagcaaaaaacctgcttggatatcagtataaatatggcggggaaacgccgaaagagggtttcgatccatcaggattgatacaatatgtgttcagtaaggctgatattcatctgccgagatctgtaaacgaccagtataaaatcggaacagctgtaaaaccggaaaacctgaagccgggtgatattttgtttttcaagaaagagggaagcaccggcactgttccgacacatgacgccctttatatcggagacggccaaatggttcacagtacacagtcaaaaggggttatcatcaccaattacaaaaaaagcagctattggagcggaacttatatcggggcgagacgaatcgctgccgatccggcaacggctgatgttcctgtcgttcaggaggccgaaaaatatatcggtgtcccatatgtgtttggcggaagcacgccgtcagagggctttgattgctcggggcttgtgcaatatgtgtttcaacaggcactcggcatttatctaccgcgatcagccgaacagcagtgggcagtgggcgagaaggtagcccctcagaacataaagcctggtgatgtcgtctatttcagcaatacgtataaaacgggaatttcacatgcaggcatttatgcgggcgcaggcaggttcattcaggcaagccggtcagaaaaagtaaccatttcctatttgtcagaggattactggaaatcgaagatgacgggtattcgccgatttgacaacctgacaatcccgaaagaaaatccgattgtttccgaagcgacgctttatgtcggagaagtgccttacaaacagggcggagtaacacctgagacgggatttgatacagctggatttgtccaatatgtataccagaaagcagccggtatttccctgcctcgatacgcaacaagccagtacaatgccggaactaagattgagaaggcggacctgaagccgggagacattgtgttctttcaatcaacaagcttaaatccctccatctatatcggaaacggacaagttgttcatgtcacattatcaaacggcgtgaccattaccaatatgaacacgagcacatattggaaggataaatacgcaggaagtatacgggtgcaataa

SEQ ID NO: 9 - protein, 382 aa, Bacillus subtilis
MKKQLTFQEKLLKLTKQQKKKTNLHVFIALPIVFCLMFVCILTGKAETPSVKRNADDLVSASFVGDIMMGRNVEKVTKHNGTESVFRYAKPFFEASDYVSGNFENPVTYKKNYKEAEKNIHLQSNKDAVKVLKDMNFTVLTAANNHAMDYGPQGMRDTVEEFSKQNLELVGAGLTLKEAEENISYQDVNGVKIATLGFTDVSGKGFAAKRNAPGVLPADPELFIPMISKAKKNADLVIVQTHWGQEYDNDPNDRQRQLARAMSDAGADIIVGHHPHVLEPIEMYHGTVIFYSLGNFVFDQGWTRTRDTALVQYHLQKNGTGRFEVTPMNIHEATPAPVKKGSINHKTIIRELTKESNFKWSVKDGKLTFDVDHSDILKKKAE

SEQ ID NO: 10 - protein, 393 aa, Bacillus subtilis
MWLLIIACAAVLIIGIIEKRRHQKNIDALPVRVNINGIRGKSTVTRLTTGILMEAGYKTVGKTTGTDARMIYWDTPEEKPIKRKPQGPNIGEQKEVMKETVERGANAIVSECMAVNPDYQIIFQEELLQANIGVIVNVLEDHMDVMGPTLDEIAEAFTATIPYNGHLVITDSEYTDFFKEKAAERNTEVIIADNSKITDEYLRKFEYMVFPDNASLALGVAQALGIDEETAFKGMLNAPPDPGAMRILPLLSTKEPGHFVNGFAANDASSTLNIWKRVKEIGYPTDEPIVIMNCRADRVDRTIQFANDVLPYIKTKELILIGETTEPIVRAYEEGKIPADTLHDLEYKSTDEIMDVLKTRMQNRVIYGVGNIHGSAEPLIEKIQEYKVKQLVS

SEQ ID NO: 11 - protein, 149 aa, Bacillus subtilis
MFGSDLYISLILGVLISLIFAEKTGIVPAGLVVPGYLGLVFNQPVFILLVLLVSLLTYVIVKYGLSRFMILYGRRKFAAMLITGICLKIALDFLYPIVPFEISEFRGIGIIVPGLIANTIQKQGLTITFASTLFLSGATFAIMFAYYLI

SEQ ID NO: 12 - protein, 411 aa, Bacillus subtilis
MLTSWRKYILAGLMICLVAPAVTRTEIAEADSQVSALMVSDAQKLVGNKYVYGGDEPKDGFDPSGLIQYLFSRQNIHLPRTVSDQWKVGAAVKENELLPGDIVFFKKSDSLQTAPVQDGLYIGNGEMIHSSPSEGVTVTSFQKSNYWMNLYLGAKRITKDPELADNPIVQEAARYLDIPYVFGGSTPEEGFDCSGLVQYVFENKLHIYLPRSAEQQWLVGEKIKLSSIKPGDVIYFSDTYKKGISHAGIYAGEGRFIQASRSAKVTISYLSEDYWKKHYTGVRRFSNLAISKDNPVVSTAADYIGISYLKGGASPETGFDTAGFVQYVYQKAKGISLPRYAEKQMQAGAPVSKQDLKPGDLVFFKAESLNPAIYIGNGQVIHVTLSAGVTITNMNTSAYWKDKYAGSIRIP

SEQ ID NO: 13 - protein, 55 aa, Bacillus subtilis
MKFVKAIWPFVAVAIVFMFMSAFKFNDQLTDQEKQKIDMEMNKIQQQEEPVNANK

SEQ ID NO: 14 - DNA, 168 bp, Bacillus subtilis
  source 1..168: mol_type = other DNA
atgaaatttgtcaaagccatctggccgtttgttgccgtagccatcgtgttcatgtttatgtcagcttttaaattcaatgatcagctgacagatcaggaaaaacagaagattgatatggaaatgaataaaatccagcagcaggaagaaccggtaaacgccaataaataa

SEQ ID NO: 15 - DNA, 25 bp, synthetic construct
  source 1..25: mol_type = other DNA
ggattaaaatcaagaactgctcttg

SEQ ID NO: 16 - DNA, 24 bp, synthetic construct
  source 1..24: mol_type = other DNA
gcttccaaaaggttctctaggtcg

SEQ ID NO: 17 - DNA, 55 bp, synthetic construct
  source 1..55: mol_type = other DNA
cttttttcatattggtaacctcctttttattaacgttttgagaactgaggtgcac

SEQ ID NO: 18 - DNA, 44 bp, synthetic construct
  source 1..44: mol_type = other DNA
taaaaaggaggttaccaatatgaaaaaagaactgagctttcatg

SEQ ID NO: 19 - DNA, 47 bp, synthetic construct
  source 1..47: mol_type = other DNA
gctcttctggtggagtctatccccgattatttagattttagtttgtc

SEQ ID NO: 20 - DNA, 49 bp, synthetic construct
  source 1..49: mol_type = other DNA
gctcttctggtggagtctatccttaaaacgtcagttttccgtcttctac

SEQ ID NO: 21 - DNA, 50 bp, synthetic construct
  source 1..50: mol_type = other DNA
gctcttctggtggagtctatccttacgtcagttttccgtcttctactttc

SEQ ID NO: 22 - DNA, 51 bp, synthetic construct
  source 1..51: mol_type = other DNA
gctcttctggtggagtctatccttacagtgcactgtctcttgttctcgtcc

SEQ ID NO: 23 - DNA, 50 bp, synthetic construct
  source 1..50: mol_type = other DNA
gctcttctggtggagtctatccttatttcgcatcacttaagctgtatccc

SEQ ID NO: 24 - DNA, 51 bp, synthetic construct
  source 1..51: mol_type = other DNA
gctcttctggtggagtctatccttaggctgagagtacgtcgtcagaatacg

SEQ ID NO: 25 - DNA, 49 bp, synthetic construct
  source 1..49: mol_type = other DNA
gctcttctggtggagtctatccttagtcagaatacgttttgaccttcgg

SEQ ID NO: 26 - DNA, 52 bp, synthetic construct
  source 1..52: mol_type = other DNA
gctcttctggtggagtctatccttaagaatacgttttgaccttcggcgtttc

SEQ ID NO: 27 - DNA, 53 bp, synthetic construct
  source 1..53: mol_type = other DNA
gctcttctggtggagtctatccttacggcgtttccgcttttcccgcccacatg

SEQ ID NO: 28 - DNA, 52 bp, synthetic construct
  source 1..52: mol_type = other DNA
gctcttctggtggagtctatccttaagcgaacataaggacaaaaacgatcgg

SEQ ID NO: 29 - DNA, 40 bp, synthetic construct
  source 1..40: mol_type = other DNA
ggatagactccaccagaagagccaggtcgatatgaacagc

SEQ ID NO: 30 - DNA, 41 bp, synthetic construct
  source 1..41: mol_type = other DNA
ccaggatgtagtatccttccgtctctcccaaagttgatccc

SEQ ID NO: 31 - DNA, 46 bp, synthetic construct
  source 1..46: mol_type = other DNA
cggaaggatactacatcctggctcaaaacgttaattttacgttttc

SEQ ID NO: 32 - DNA, 25 bp, synthetic construct
  source 1..25: mol_type = other DNA
ctttgctattatgagctactaacgc

SEQ ID NO: 33 - DNA, 25 bp, synthetic construct
  source 1..25: mol_type = other DNA
gttcgataacctgctgttcaacagc

SEQ ID NO: 34 - DNA, 30 bp, synthetic construct
  source 1..30: mol_type = other DNA
ggagtgtcaagaatgtttgcaaaacgattc

SEQ ID NO: 35 - DNA, 29 bp, synthetic construct
  source 1..29: mol_type = other DNA
tcaatggggaagagaaccgcttaagcccg

SEQ ID NO: 36 - DNA, 25 bp, synthetic construct
  source 1..25: mol_type = other DNA
gtgataaagatgaaatttgtcaaag

SEQ ID NO: 37 - DNA, 28 bp, synthetic construct
  source 1..28: mol_type = other DNA
cttacattaaattaagtagtaaacaaac

SEQ ID NO: 38 - DNA, 25 bp, synthetic construct
  source 1..25: mol_type = other DNA
aatttaatgtaaggtgtgtcaaacg

SEQ ID NO: 39 - DNA, 25 bp, synthetic construct
  source 1..25: mol_type = other DNA
acaaatttcatctttatcactccga

SEQ ID NO: 40 - DNA, 52 bp, synthetic construct
  source 1..52: mol_type = other DNA
cgtttgacacaccttacattaaattaagtagtaaacaaacatgatagcaaag

SEQ ID NO: 41 - DNA, 50 bp, synthetic construct
  source 1..50: mol_type = other DNA
tcggagtgataaagatgaaatttgtcaaagccatctggccgtttgttgcc

SEQ ID NO: 42 - DNA, 30 bp, synthetic construct; identical to SEQ ID NO: 34
  source 1..30: mol_type = other DNA

SEQ ID NO: 43 - DNA, 30 bp, synthetic construct
  source 1..30: mol_type = other DNA
attgctgtttcatttggttctggcaggacc

SEQ ID NO: 44 - DNA, 30 bp, synthetic construct
  source 1..30: mol_type = other DNA
caatggggaagagaaccgcttaagcccgag

SEQ ID NO: 45 - DNA, 30 bp, synthetic construct
  source 1..30: mol_type = other DNA
acgtaatcaaagccaggctgattctgaccg